European Patent Specification EP 3 467 509 B1, published November 26, 2025. Title: CNS Antigen-Specific B Cell, T Cell, and Antibody Assays and Their Uses in Diagnosis and Treatment of Multiple Sclerosis. Applicant: Cellular Technology, Ltd. Application EP 12782351.6. The sequence listing filed with the application follows.

SEQUENCE LISTING (7 sequences)

SEQ ID NO: 1 - protein, 247 aa, Homo sapiens
MASLSRPSLPSCLCSFLLLLLLQVSSSYAGQFRVIGPRHPIRALVGDEVELPCRISPGKNATGMEVGWYRPPFSRVVHLYRNGKDQDGDQAPEYRGRTELLKDAIGEGKVTLRIRNVRFSDEGGFTCFFRDHSYQEEAAMELKVEDPFYWVSPGVLVLLAVLPVLLLQITVGLVFLCLQYRLRGKLRAEIENLHRTFDPHFLRVPCWKITLFVIVPVLGPLVALIICYNWLHRRLAGQFLEELRNPF

SEQ ID NO: 2 - protein, 20 aa, Homo sapiens
SSYAGQFRVIGPRHPIRALV

SEQ ID NO: 3 - protein, 197 aa, Homo sapiens
MASQKRPSQRHGSKYLATASTMDHARHGFLPRHRDTGILDSIGRFFGGDRGAPKRGSGKVPWLKPGRSPLPSHARSQPGLCNMYKDSHHPARTAHYGSLPQKSHGRTQDENPVVHFFKNIVTPRTPPPSQGKGRGLSLSRFSWGAEGQRPGFGYGGRASDYKSAHKGFKGVDAQGTLSKIFKLGGRDSRSGSPMARR

SEQ ID NO: 4 - protein, 247 aa, Homo sapiens
MGLLECCARCLVGAPFASLVATGLCFFGVALFCGCGHEALTGTEKLIETYFSKNYQDYEYLINVIHAFQYVIYGTASFFFLYGALLLAEGFYTTGAVEQIFGDYKTTICGKGLSATVTGGQKGRGSRGQHQAHSLERVCHCLGKWLGHPDKFVGITYALTVVWLLVFACSAVPVYITFNTPWNAFPGKVCGSNLLSICKTAEFQMTFHLFIAAFVGAAATLVSLLTFMIAATYNFAVLKLMGRGTKF

SEQ ID NO: 5 - protein, 13 aa, Homo sapiens
HCLGKWLGHPDKF

SEQ ID NO: 6 - protein, 8 aa, Synthetic
LLGGLEDP

SEQ ID NO: 7 - protein, 452 aa, Synthetic
MASQKRPSQRHGSKYLATASTMDHARHGFLPRHRDTGILDSIGRFFGGDRGAPKRGSGKVPWLKPGRSPLPSHARSQPGLCNMYKDSHHPARTAHYGSLPQKSHGRTQDENPVVHFFKNIVTPRTPPPSQGKGRGLSLSRFSWGAEGQRPGFGYGGRASDYKSAHKGFKGVDAQGTLSKIFKLGGRDSRSGSPMARRLLGGLEDPMGLLECCARCLVGAPFASLVATGLCFFGVALFCGCGHEALTGTEKLIETYFSKNYQDYEYLINVIHAFQYVIYGTASFFFLYGALLLAEGFYTTGAVEQIFGDYKTTICGKGLSATVTGGQKGRGSRGQHQAHSLERVCHCLGKWLGHPDKFVGITYALTVVWLLVFACSAVPVYITFNTPWNAFPGKVCGSNLLSICKTAEFQMTFHLFIAAFVGAAATLVSLLTFMIAATYNFAVLKLMGRGTKF